European Patent Specification EP 4 301 880 B1, published July 15, 2026. Title: METHOD FOR DETECTION OF SARS-CoV-2 MUTATIONS. Applicant: SEEGENE, INC. The sequence listing filed with the application follows.

SEQUENCE LISTING (5 sequences)

SEQ ID NO: 1 - DNA, 102 bp, Artificial Sequence
  oligonucleotide comprising mutation-discriminating site for HV69/70 del
ctcaggacttgttcttacctttcttttccaatgttacttggttccatgctatctctgggaccaatggtactaagaggtttgataaccctgtcctaccattta

SEQ ID NO: 2 - DNA, 102 bp, Artificial Sequence
  oligonucleotide comprising mutation-discriminating site for Y144 del
tgttattaaagtctgtgaatttcaattttgtaatgatccatttttgggtgtttaccacaaaaacaacaaaagttggatggaaagtgagttcagagtttattc

SEQ ID NO: 3 - DNA, 103 bp, Artificial Sequence
  oligonucleotide comprising mutation-discriminating site for E484K
atatttcaactgaaatctatcaggccggtagcacaccttgtaatggtgttaaaggttttaattgttactttcctttacaatcatatggtttccaacccactaa

SEQ ID NO: 4 - DNA, 103 bp, Artificial Sequence
  oligonucleotide comprising mutation-discriminating site for N501Y
aaggttttaattgttactttcctttacaatcatatggtttccaacccacttatggtgttggttaccaaccatacagagtagtagtactttcttttgaacttct

SEQ ID NO: 5 - DNA, 103 bp, Artificial Sequence
  oligonucleotide comprising mutation-discriminating site for P681H
tacccattggtgcaggtatatgcgctagttatcagactcagactaattctcatcggcgggcacgtagtgtagctagtcaatccatcattgcctacactatgtc